European Patent Specification EP 4 092 044 B1, published September 25, 2024. Title: Recombinant vector comprising codon-optimized TIF1r polynucleotide and use the same. Applicant: Neo-Gene-Pharm Inc. The sequence listing filed with the application follows.

SEQUENCE LISTING (5 sequences)

SEQ ID NO: 1 - DNA, 3385 bp, Artificial Sequence
  codon optimization of TIF1gamma full sequence
catggccgagaacaaaggcggcggagaagctgaatctggcggaggcggatctggatctgctcctgttacagctggtgccgctggacctgctgctcaagaagcagaacctcctctgacagccgtgctggtggaagaagaagaggaagaaggcggcagagctggcgctgaaggcggagctgctggaccagatgatggcggagttgccgctgcctctagtggatctgcacaggctgcatctagccctgccgcctctgttggaacaggtgttgctggcggagccgtgtctacaccagctccagcaccagcaagtgctccagctcctggaccttctgcaggacctccacctggacctccagcttctctgctggatacctgtgccgtgtgtcagcagagcctgcagagcagaagagaggccgagcctaagctgctgccttgcctgcacagcttctgcctgagatgtctgcccgagcctgagagacagctgagcgttccaattcctggcggcagcaacggcgacattcagcaagtgggcgtgatcagatgccccgtgtgcagacaagagtgccggcagattgacctggtggacaactacttcgtgaaggacaccagcgaggcccctagcagctctgacgagaagtctgagcaagtgtgcacctcctgcgaggacaatgcctctgccgtgggcttctgtgtggaatgtggcgagtggctgtgcaagacctgtatcgaggcccaccagagagtgaagttcaccaaggaccacctgatccggaagaaagaagatgtgtccgagagcgtgggcgcctctggacaaagacctgtgttctgccccgtgcacaagcaagagcagctgaagctgttctgcgagacatgcgaccggctgacctgcagagattgccagctgctcgaacacaaagagcacagataccagtttctggaagaggcctttcagaaccagaagggcgccatcgagaacctgctggccaaactgctggaaaagaaaaactacgtgcacttcgccgccacacaggtgcagaaccggatcaaagaagtgaacgagacaaacaagcgggtcgagcaagagatcaaggtggccatcttcaccctgatcaacgagatcaacaagaagggcaagagcctcctgcagcagctggaaaacgtgaccaaagaacggcagatgaagctgcttcagcagcagaacgacatcaccggcctgagcagacaagtgaagcacgtgatgaatttcaccaactgggccattgccagcggcagctctacagccctgctgtactccaagcggctgatcaccttccagctgagacacatcctgaaggccagatgcgatcctgtgcctgccgccaatggcgctatcagattccactgcgaccccaccttttgggccaagaacgtcgtgaacctgggcaacctggtcatcgagagcaagcctgctcctggctacacccctaatgtggtcgttggacaggtgccacctggcaccaaccacatctctaagacccctggccagatcaacctggctcagctcagactgcagcacatgcagcagcaagtgtacgcccagaaacaccagcagctgcagcagatgcggatgcagcaacctcctgctccagtgcctaccaccaccacaaccacacagcagcaccctagacaggccgctcctcagatgctgcaacagcagcctccaagactgatcagcgtgcagactatgcagcggggcaacatgaactgcggagcctttcaggcccatcagatgagactggcccagaacgccgctagaatccctggcatccctagacacagcggccctcagtacagcatgatgcagccccatctgcagagacagcacagcaatcctggacacgccggaccttttccagtggtgtctgtgcacaataccacgatcaaccctacaagccccaccaccgccacaatggccaatgccaatagaggcccaacaagccctagcgtgacagccatcgagctgatccccagcgtgacaaaccccgagaatctgcctagcctgcctgacatccctcctatccagctcgaggatgccggctctagcagcctggataatctgctgagccggtacatcagcggctcccatcttccacctcagcctaccagcacaatgaacccatctccaggaccaagcgctctgagccctggatctagcggactgagcaacagccacacacctgtgcggcctccaagcacaagcagcacaggctctagaggaagctgtggcagcagcggaagaaccgccgaaaagaccagcctgagcttcaagagcgaccaagtgaaagtgaaacaagagcccggcaccgaggacgagatctgcagtttttctggcggcgtgaagcaagagaaaaccgaggatgggagaagatctgcctgcatgctgagcagccctgagagcagccttacacctccactgagcaccaacctgcacctggaaagcgaactggatgccctggcctctctggaaaaccacgtgaaaacagagcccgccgacatgaacgagagctgcaagcagtctggactgtccagcctggtcaacggcaagtcccctatccgcagcctgatgcacagaagcgctagaattggcggcgacggcaacaacaaggacgacgaccctaacgaggattggtgcgccgtctgtcagaacggcggagatctgctgtgttgcgagaagtgccccaaggtgttccacctgacctgccacgttccaacactgctgtctttccccagcggcgactggatctgtaccttctgtagagacatcggcaagcccgaggtggaatacgactgcgacaatctgcagcactccaaaaagggcaaaacagcccagggactgagccccgtggatcagagaaagtgcgagagactgctgctgtacctgtactgccacgagctgagcatcgagttccaagagccagtgcctgccagcattcccaactactacaagatcatcaagaaaccgatggacctgagcaccgtcaagaagaagctgcagaagaagcactcccagcactatcagatccccgacgacttcgtggctgacgtgcgcctgatctttaagaactgcgagcggttcaatgagatgatgaaggtggtgcaggtctacgccgacacacaagagattaacctgaaagccgacagcgaggtggcccaggccggaaaagctgtcgccctgtacttcgaggacaagctgaccgagatctacagcgaccggacattcgctcctctgccagagtttgagcaagaagaggacgacggggaagtgaccgaggacagcgacgaggatttcatccagcctcggcggaagagactgaagtccgatgagcggccagtgcacatcaaatga

SEQ ID NO: 2 - DNA, 857 bp, Artificial Sequence
  codon optimization of TIF1gamma N term sequence
tgtgctgtttgtcagcagagcctgcagagcagaagagaggccgagcctaagctgctgccttgcctgcacagcttctgcctgagatgtctgcccgagcctgagagacagctgagcgttccaattcctggcggcagcaacggcgacatccagcaagtgggagtgatcagatgccccgtgtgctgcaccagctgcgaggacaatgcctctgccgtgggcttctgtgtggaatgtggcgagtggctgtgcaagacctgtatcgaggcccaccagagagtgaagttcaccaaggaccacgccccgtgcacaagcaagagcagctgaagctgttctgcgagacatgcgaccggctgacctgcagagattgccagctgctggaacacaaagagcatctggaagaggcctttcagaaccagaagggcgccatcgagaacctgctggccaaactgctggaaaagaaaaactacgtgcacttcgccgccacacaggtgcagaaccggatcaaagaagtgaacgagacaaacaagcgggtcgagcaagagatcaaggtggccatcttcaccctgatcaacgagatcaacaagaagggcaagagcctcctgcagcagctcgagaacgtgaccaaagaacggcagatgaagctgctccagcagcagaacgatatcaccggcctgagccggcaagtgaagcacgtgatgaatttcaccaactgggccattgccagcggctctagcacagccctgctgtactccaagcggctgatcaccttccagctgcggcacatcctggccatccggttccactgcgaccctaccttttgggccaagaacgtggtcaacctgggcaacctggtcatcgag

SEQ ID NO: 3 - DNA, 411 bp, Artificial Sequence
  codon optimization of TIF1gamma C term sequence
tgcgccgtctgccagaacggcggagatctgctgtgttgcgagaagtgccccaaggtgttccacctgacctgccacgttccaacactgctgagcttccctagcggcgactggatctgcaccttctgccagggactgagccccgtggatcagagaaagtgcgagagactgctgctctacctgtactgccacgagctgagcatcgagttccaagagcctgtgcctgccagcattcccaactactacaagatcatcaagaaacccatggacctgagcaccgtgaagaagaagctgcagaagaagcacagccagcactatcagatccccgacgacttcgtggctgacgtgcggctgatcttcaagaactgcgagcggttcaacgagatgatgaaggtggtgcaggtctacgccgac

SEQ ID NO: 4 - DNA, 2778 bp, Artificial Sequence
  codon optimization of TIF1gamma N and C term sequence
tgtgctgtttgtcagcagagcctgcagagcagaagagaggccgagcctaagctgctgccttgcctgcacagcttctgcctgagatgtctgcccgagcctgagagacagctgagcgttccaattcctggcggcagcaacggcgacattcagcaagtgggcgtgatcagatgccccgtgtgcagacaagagtgccggcagattgacctggtggacaactacttcgtgaaggacaccagcgaggcccctagcagctctgacgagaagtctgagcaagtgtgcacctcctgcgaggacaatgcctctgccgtgggcttctgtgtggaatgtggcgagtggctgtgcaagacctgtatcgaggcccaccagagagtgaagttcaccaaggaccacctgatccggaagaaagaagatgtgtccgagagcgtgggcgcctctggacaaagacctgtgttctgccccgtgcacaagcaagagcagctgaagctgttctgcgagacatgcgaccggctgacctgcagagattgccagctgctcgaacacaaagagcacagataccagtttctggaagaggcctttcagaaccagaagggcgccatcgagaacctgctggccaaactgctggaaaagaaaaactacgtgcacttcgccgccacacaggtgcagaaccggatcaaagaagtgaacgagacaaacaagcgggtcgagcaagagatcaaggtggccatcttcaccctgatcaacgagatcaacaagaagggcaagagcctcctgcagcagctggaaaacgtgaccaaagaacggcagatgaagctgcttcagcagcagaacgacatcaccggcctgagcagacaagtgaagcacgtgatgaatttcaccaactgggccattgccagcggcagctctacagccctgctgtactccaagcggctgatcaccttccagctgagacacatcctgaaggccagatgcgatcctgtgcctgccgccaatggcgctatcagattccactgcgaccccaccttttgggccaagaacgtcgtgaacctgggcaacctggtcatcgagagcaagcctgctcctggctacacccctaatgtggtcgttggacaggtgccacctggcaccaaccacatctctaagacccctggccagatcaacctggctcagctcagactgcagcacatgcagcagcaagtgtacgcccagaaacaccagcagctgcagcagatgcggatgcagcaacctcctgctccagtgcctaccaccaccacaaccacacagcagcaccctagacaggccgctcctcagatgctgcaacagcagcctccaagactgatcagcgtgcagactatgcagcggggcaacatgaactgcggagcctttcaggcccatcagatgagactggcccagaacgccgctagaatccctggcatccctagacacagcggccctcagtacagcatgatgcagccccatctgcagagacagcacagcaatcctggacacgccggaccttttccagtggtgtctgtgcacaataccacgatcaaccctacaagccccaccaccgccacaatggccaatgccaatagaggcccaacaagccctagcgtgacagccatcgagctgatccccagcgtgacaaaccccgagaatctgcctagcctgcctgacatccctcctatccagctcgaggatgccggctctagcagcctggataatctgctgagccggtacatcagcggctcccatcttccacctcagcctaccagcacaatgaacccatctccaggaccaagcgctctgagccctggatctagcggactgagcaacagccacacacctgtgcggcctccaagcacaagcagcacaggctctagaggaagctgtggcagcagcggaagaaccgccgaaaagaccagcctgagcttcaagagcgaccaagtgaaagtgaaacaagagcccggcaccgaggacgagatctgcagtttttctggcggcgtgaagcaagagaaaaccgaggatgggagaagatctgcctgcatgctgagcagccctgagagcagccttacacctccactgagcaccaacctgcacctggaaagcgaactggatgccctggcctctctggaaaaccacgtgaaaacagagcccgccgacatgaacgagagctgcaagcagtctggactgtccagcctggtcaacggcaagtcccctatccgcagcctgatgcacagaagcgctagaattggcggcgacggcaacaacaaggacgacgaccctaacgaggattggtgcgccgtctgtcagaacggcggagatctgctgtgttgcgagaagtgccccaaggtgttccacctgacctgccacgttccaacactgctgtctttccccagcggcgactggatctgtaccttctgtagagacatcggcaagcccgaggtggaatacgactgcgacaatctgcagcactccaaaaagggcaaaacagcccagggactgagccccgtggatcagagaaagtgcgagagactgctgctgtacctgtactgccacgagctgagcatcgagttccaagagccagtgcctgccagcattcccaactactacaagatcatcaagaaaccgatggacctgagcaccgtcaagaagaagctgcagaagaagcactcccagcactatcagatccccgacgacttcgtggctgacgtgcgcctgatctttaagaactgcgagcggttcaatgagatgatgaaggtggtgcaggtctacgccgac

SEQ ID NO: 5 - DNA, 470 bp, Artificial Sequence
  human TGF promoter
gtcgactgacagaccctcttctcctaccttgtttcccagcctgactctccttccgttctgggtccccctcctctggtcggctcccctgtgtctcatcccccggattaagccttctccgcctggtcctctttctctggtgacccacaccgcccgcaaagccacagcgcatctggatcacccgctttggtggcgcttggccgccaggaggcagcaccctgtttgcggggcggagccggggtgcccgccccctttcccccagggctgaagggacccccctcggagcccgcccacgcgagatgaggacggtggcccagcccccccatgccctccccctgggggccgcccccgctcccgccccgtgcgcttcctgggtggggccgggggcggcttcaaaaccccctgccgacccagccggtccccgccgccgccgcccttcgcgccctgggccatctccctcccacctccctccg